European Patent Application EP 4 170 035 A1, published April 26, 2023. Title: APPLICATION OF METHIONINASE GENE THERAPY IN TREATMENT OF MALIGNANT TUMOR. Applicant: Guangzhou Sinogen Pharmaceutical Co., Ltd. The sequence listing filed with the application follows.

SEQUENCE LISTING (3 sequences)

SEQ ID NO: 1 - DNA, 1263 bp, Artificial Sequence
  MEGL
atgcgcgactcccataacaacaccggtttttccacacgggccattcaccacggctacgacccgctttcccacggtggtgccttggtgccaccggtgtaccagaccgcgacctatgccttcccgactgtcgaatacggcgctgcgtgcttcgccggggaggaggcggggcacttctacagccgcatctccaaccccaccctggccttgctcgagcaacgcatggcctcgttggagggtggtgaggcgggattggcgctggcgtcggggatgggagccattacttcgaccctctggaccctgctgcggcctggtgatgagctgatcgtggggcgcaccttgtatggctgcacctttgcgttcctgcaccatggcattggcgagttcggggtcaagatccaccatgtcgaccttaacgatgccaaggccctgaaagcggcgatcaacagcaaaacgcggatgatctacttcgaaacaccggccaaccccaacatgcaactggtggatatagcggcggtcgtcgaggcagtgcgggggagtgatgtgcttgtggtggtcgacaacacctactgcacgccctacctgcagcggccactggaactgggggcagacctggtggtgcattcggcaaccaagtacctcagtggccatggcgacatcactgcgggcctggtggtggggcgcaaggctttggtcgaccgcattcggctggaagggctgaaagacatgaccggggcagccttgtcaccgcatgacgctgcgttgttgatgcgcggcatcaagaccctggcgctgcgcatggaccggcattgcgccaacgccctggaggtcgcgcagttcctggccgggcagccccaggtggagctgatccactacccgggcttgccgtcgtttgcccagtacgaactggcacagcggcagatgcgtttgccgggcgggatgattgcctttgagctcaagggcggtatcgaggccgggcgcggcttcatgaatgccctgcagctttttgcccgtgcggtgagcctgggggatgccgagtcgctggcacagcacccggcgagcatgacgcactccagttacacgccacaagagcgggcgcatcacgggatatcagaggggctggtgaggttgtcagtggggctggaggatgtggaggacctgctggcagatatcgagttggcgttggaggcgtgtgcagactacaaagaccatgacggtgattataaagatcatgatatcgattacaaggatgacgatgacaagtga

SEQ ID NO: 2 - DNA, 24 bp, Artificial Sequence
  MEGL-F
cacttctacagccgcatctccaac

SEQ ID NO: 3 - DNA, 23 bp, Artificial Sequence
  MEGL-R
gaccaccacaagcacatcactcc